European Patent Application EP 4 368 627 A1, published May 15, 2024. Title: COMPOSITION COMPRISING NUCLEIC ACID OLIGOMER. Applicant: SUMITOMO CHEMICAL COMPANY, LIMITED. The sequence listing filed with the application follows.

SEQUENCE LISTING (2 sequences)

SEQ ID NO: 1 - RNA, 103 nt, Artificial Sequence
  Synthetic oligonucleotide
  modified_base (2)..(2), (100)..(102): phosphorothioate derivative of uracil
  modified_base (1)..(1), (3)..(3): phosphorothioate derivative of adenosine
nnnacucaauuuguaaaaaaguuuuagagcuagaaauagcaaguuaaaauaaggcuaguccguuaucaacuugaaaaaguggcaccgagucggugcuuunnnu

SEQ ID NO: 2 - RNA, 67 nt, Artificial Sequence
  Synthetic oligonucleotide
  modified_base (4)..(4), (6)..(6), (14)..(14), (25)..(25), (37)..(37), (42)..(46): am
  modified_base (2)..(2), (7)..(7), (22)..(22), (41)..(41), (47)..(47), (55)..(55),(61)..(61), (63)..(63): gm
  modified_base (29)..(29), (38)..(38), (53)..(54): cm
  modified_base (5)..(5), (39)..(40), (48)..(48), (62)..(62): um
  modified_base (23)..(23), (28)..(28): phosphorothioate derivative of cytosine
  modified_base (24)..(24), (27)..(27): phosphorothioate derivative of uracil
  modified_base (26)..(26): phosphorothioate derivative of guanine
  modified_base (1)..(1): phosphorothioate derivative of 2'-O-methyladenosine
  modified_base (2)..(2): phosphorothioate derivative of 2'-O-methylguanosine
  modified_base (3)..(3), (64)..(64): phosphorothioate derivative of 2'-O-methylcytidine
  modified_base (65)..(66): phosphorothioate derivative of 2'-O-methyluridine
nnnnnnncaaguunaaauaagnnnnnnnnguuaucannnnnnnnnnnnggcannnagucgnnnnnnu